European Patent Specification EP 3 488 013 B1, published September 6, 2023. Title: Methods of diagnosis Alzheimer's disease. Applicant: EPFL. The sequence listing filed with the application follows.

SEQUENCE LISTING (5 sequences)

SEQ ID NO: .1 - DNA, 31 bp, Homo sapiens
aaaagaattcgccaccatggctcagcggtgc

SEQ ID NO: .2 - DNA, 28 bp, Homo sapiens
caagggatccagatgtcgggaggaaggg

SEQ ID NO: .3 - DNA, 36 bp, Homo sapiens
agtaggtacccttagcttagccatgtcatagccttc

SEQ ID NO: .4 - DNA, 40 bp, Homo sapiens
cgacgcgtcgatattggtttactctcgtatccttaaaaag

SEQ ID NO: .5 - DNA, 63409 bp, Homo sapiens
aaaaaagtatctctgaaaattattttaaatattgagttgagcaaaaacgctaagttaaacattttggctgtttttcctaaaatgttttaaacagctaaaaatcaatgtgtatggaatgtattcaccattgaggagatattaaaaaaaacctgaccatcttcacactgaatactaggcaagaaagattagtaccatggaaaaaaaatgctagttttgtattcagatctgagctcaaaccttagctctgctatcatagctctgtaactgtaacatattctttaagcttgttttgtcatgttacatggtgataaagaaaaatacttgttacagggttgtaataaggataaaacaaagtgaaaacctctagcacagttcctgactgcattttttctcaatgtttgttgaaaatgaaaacattttaaacatttaaaatgaaaattttaaacactgtaattttcaggtaattaattacatgtatgttgagcaaaagtgaatacttttcttataaaagtaactttccggccgggcgcggtagttcacgcctgtaatcccagcactttgggaggctgaagtgggtggatcgcctgaggtcaagagttcgagaccagcctggccaacatggtgaaaccctgtccctactaaaaatacaaaagttagctgggtgtggtagtgggcacctgtaattccagctactctgaggctgaggcaggagaatcacttgaacccgggaggtggaggttgcaatgagccgagattgcaccattgcactcccgcctgggcaacaagagggaaatcccatctcaaataaataaataactcccccattattcaggcattgtaaattatgtatctttgatggcatgtctttgaaggaattatgtctttttagaggaaactgacaggtaattttaaaaagtatagatccaaggttaataaactcacttctctctctctctctctcacacacacacacacacacacacacacacacacactagagaataagagaatgagccagtctcatctacaaccatattaaacttgtgtcttcatgtgcacatttggtaacacattttgaactaccttgaattttcaagtttctagtttttctctttagctgaggacttcttgaaaccaattgttttgggggagagaatatttttagaatccaggcatggcccaaacaattctctttgaaaagaaagcaaactggaatcctgggaaagccgttaattctcaacactacttataaacatgacaaacaataaaataaattctataacaacttgtaagagcttatgttttcacatctaaattttcaatggtaaggttccttacaatctcaagtgttaaacaaaaggtatcaagcacacttaggttacaaggagaagcaaaaagattggtttgagcaacctggatcactttcaataagggaggaggatctctggagagtgtaacagctgaatttcaagaaatctggtttctagtttgggcaagtcagtaaatctgagctttctttctcacctcttacaagtaatggcattttccttccttcctcacaaagttgactcatgaaagcacttaaaaaagttaaaaatgttacatactatgttctttaatcagcactaataacattaatattgatcgggcagaaggtacagcgatcatgcgggtggggaccagaattgggaattgggaattgggaaatctaggttctcagcccaacatttgcacctgctagttcgtgatgcaaggcacctcacttatccaggtccccattaaactaggtttaataaagtgagtttgcctaaacctcttcctagctccaaggctaattttaagctattaatttgaatccaaggcctaaaatatttgagctctcatttaacagtcggccactgcaaagggtaaagacagcaatcttgtatgaacaaagttaaacataacgtgctagacacaggtctttgcaaaaccatgcagtagccaataggtccaccataccacccttcatttggaaattgatgctaaggtgccataggtacatttccaaatgctcttaaaatgtttaggttcatattaaaataaaaatggatatttatggtacaatgagaaccagaaaaactgcaaaattatacacaggcctaagggcagaaataccccaaaagacgacacagtgacaatattttccaacttgtgcttttttgtttttaaaacaaggctgatgattctgaaatcaggtcaatgtctatcacttttttcgttgatgttaaatgcactaagggaatatagattcttcaattatactttgaaacaacatcatttccctaagtcaggacttttttattgcaaaatttaacaaaccaccaaactcaagtttaattatttctgctttattattggtcatgaataaagacttcttttaaaaaataattacaaagaatttatgactaaaatatactccgtaaccaacttgctctgaaattaataatttgaaaatggcaaagaaaaaaaaaaacagcccacaacatattaacttcactcttcaattaggggaaataaacaaggtcaaaattagtttaaacaacatactgagtaataaaaaagttgtgcagaagtcccaatgcctccaaaaaactgatagaatgtgcttaatatatatatccccacatggtaacataaaaaatccaagttttccagtaaaaatgttctgttcatgttccaatacctaaatctgggaaaacaaattcaggcagatgagataagaacgtcaccacaataaaataaagtcatcaaaacttagtgaactaaaatttaaaaggtagaggaattatttttcctaatttgacctaatttgaccacacagtaattacttccagaagacaaaagatccaatccaggtaaaataaatctttattttattattttacctgatcctaaagaaaatattctacgtgagttgatggatacattggtcaagttttatgccaaaaaaattacgcaaactatactctgaaagagctatccagactccttgccaaaaggccagcataactttcagagtagagatcgtgagttaccacagatgctgattgaaacagagctaacagcagctttctcctcattcccaccccgtgtgtaggagtacgcagtctcataccaccaccagttggaggatgatctagtctggagacagaacggtgtagaacaaaacccttgccagggtcccaaacctctctttagaactctaattaaaggtacttccgtttcccacacaacttggaatgaaggggaagcaacgactgttaaaacatttaaaaactaagcctttatctatttatttagaaaacacactatgcaaagaagccaattccttacattaaaaatatttatttgcaacagctctcctttttaaggcctcaacagattggactaaaccacacccctccataaatggcacattccatacaatagcctggagaatggcataggacgattccaccgacagctgggggaatagcaaacttgttgaaattccgagaatgaagtctgatggttacccgaacctagcccttttattactaaagtcactcggggacaagagggttacaaaaatatcccgagacgcgtacgcgggtgagagtggaacgagaaccacacgggatttgggccgtgctgttaacccgcacctccctgagtacggacatttccccgaggaaggacatttctagtcggagagaaagagcgaactttggggttaactctctcaaaactctgaggtggggagagaggcagcagcccattattttccaggatccagtcccgaactctcacttttgcccggggggaaaaaaacgggtcccgcccacgctcggcccgatccgggaggcggggcctgcagcgaccccgaaggacagaggcggggccggttggcagtgctgcccctccccctttgccaggaacacccccgtccgctacagagagggctcagggcccccacccccgcgccagtcgctgggggaaggggcaatacgggtgcctccgcccctcctcgctgaaggtggggagtggagctcgagtccgcccgcctccccgcgctggctccaaggggacggccccgaggaggtggggcctcttgggggcgctgacttcacacccctccccctccggccgctggcggctcagggacaccccgcccgctctagtgcggtgggtgggggaggcagctgagcagaccggagccctgcagcggcgcggggcggggaggggcgcgcgcacgggcgcgcagccaccacccccgcgcgccagcagggccccccacgctcaagggtgcgcgcgggccccgaaagggaggaggccgcgcgcggcaccggggatggcggactctagccttctgtcccccactcttttcaccactcgcccccatccccctccaacccgctccaggcctcagactccgcactgacctgacaggccgcgacatgttcgctgtcgaaacaggaccgagtcgagaagccaaagaccaggaccccccccaccccgcgcgctcggcgccccaccccccccgaacttcagccgatgggaccgctgctgccgaaccccgagctgctggcttctcaaactccgctgctctttggttcagggctcctggaacagacgagccccccgctcccccgtctcttcaaaatggatgaatcaaaccagccgaaaatgcgccaaagccgccgtgcaaccaaacccactagggtttgtgcgctcctccccaacacgcctgctcattggagacttctgccagatgcgcccagatcattagtccgtttgaatcatcacgtcttccaggccccgccctgctctctgataggctccaccttcaccgtgggggtcctgttagtcaagatgctctgagagcgcacggccgcaaaacaaaaatggtcgctgcttagcccgccccctggtttccactccagagttgcagattcgtctggggtcgtatcttagaaagactagaaaaaaagatttatgtagggttcagcgttgctcagtgttagtttaatggtgtttcatctcgtctgccttgatcaccttgaaaatcctctaatagcaaaacccgtgggagaggcagcagattcgtcactgcggggctgctacagaattggagggaaattccttaggttcaaaaaatttgaccttaaacctacaagccccttaccctggcttcggcattaaccctcagggaccaaatgaggctgctggagtagagaggcaggatcataatcaaggaatatcttcacccccaattaccattctccattctggaccttgagatccacttcagggtcattaaagtcccagtctggtgcattactattttaagaaaagagtcaggtgtacaataactaagagcatgagctcaggggccacaaggtatttcaggtggaatcccaggtccactacttaatggtggtataactttccttctctgtgcctcagttttctcatctgtaaaatgggaaacaagggtacctaactgcataggcttattagtattaaatgagttgatatatctatcaaaagtctttaggatagtctctggctcacagtaagtgctacgtaagtgttaaatccaagttttaaaagatgattccgtccctgggtagagatgggtggagctggctcaagaccctatgaattctattgatttacccttgcactttgaaaaacaaaacaaagactcttcgaagtcatataactgaaagtaacgcacatcatttcacttaaatccgtgagcatttgttggatgcctaatactctcaaaggcagagctcaggattcctatgtgaatggctaaggctgagtctgctatcgaaaatagacgtcaatccctgtcacagtcaaagcgatcatttttgtttggtggctgtgcgctctcagagcatcttgactaacaggaccccacggtgaaggtggggcctatcagagagtagggtggggcctggaagacgtgatgattcaaacggactaatgatctgggcgcatctggcagaagtctccaatgagcagtcagttaacaaccaattgaagatacactttccaaacaacaacaacaaaaaacacaccacatctgcctcctgaaagtctccctttgtaaaatctggcttcccaaaaagaagagaatagcacagtccaccagtgaagcattaaacaaattaatatcttttgtctcttccatgtcattccaccctctgtccctcttatttttatttttaatttttattttttcgagacggagtctcactcactatgctccccaggctggattgcagtggcacgatctctgcacactgaaacttccaccacccgggttcaagcgattctcctgcctcagcctcccaagtagctgggattacaggcgtgctccaccatgcccagctaattttggtattttattgtggagatggggtttcaccatgttggccaggctggtcttgaactcttgacctcaagtgatctgcctgccttggcctcccaaagtgctggcattacaggagtgagccaccgcacccgtcccccgcaatttttttaaattgtggttaaaaaaaaaatacataacataaatgtaccactttaactgtctctaagtgtacagttaagtggcgttaagtacattcacattgttatgcaaccatcaccacgattcaacaccagaactttctcattttcccaaactgaaactctgtgcccattaaacactaactccccactttcccccttccccatagccgctggcaaccaccattttactttctgtctgtatgaacctgactgctctaggaatctcatgttagtgtaatcatacagtatttgtccttttgtgactggcttatttcacttagcataatggcatccaggtttatccatgttgtagcaagtgtcaaaatttcctttctcttaaaggccaaataatattccactgtatgtatatgccacattttgtttatccactcatccatcaatggacacttgggttgcttccaccttatggctattgtgaatgatgttgctgggcaagtgggagtacaaatatgtttgagtacctgctttcctttctggatatatacccagaaatggaattgctagatcatacagctattctgtttaattttttgaagaattgccgtatggattctccatcagctgtatcattttacactcctaccagcaatgtgcaagtgttccaatttccccatgtccttgccaacagtaagttttttacaatagccatcctaatgagtgtccatatacggtttttttttttttttttgaaacggagtctcgctctgttgcccaggctggagtgcagtggtgcgatctctgctcactgcaaactccgcctcccaggttcacgccattctcctgcctcagcctcccaagtagctgagactacagatgcccgccaccacgcctggctaatttttgtatttttagtacagacggagtttcattacgttggccaggctggtctcaaactcctgacctcaggtgatccacccgcctcggcctcccaaagtgctgggattacaggcatgagccaccacgcccagccttttttttttttttagatagagtctagccctgtcacctggtctggctcactgcagcctctacctcccgggttcaagcaattctcctgccttagcctcagagtagctgggattacaggcatgcgccaccacacctggctttttgtatttttagtagagacggggtttcactatgtttgccaggctggtctcgaactcctgacctcaagtgatccacccacctcagcctcccaaagtgctgggattacaggcgtgagccaccgcgcccggctccatatatgttttgactaagtgtattaccatccccactattgtcagaatgccagggcagaaacttgggtggcagagtgatcaccaagtggctttggtggaggctcttttattaggccaaattgttattattttagtaaacatcattatttggtattgtgagatggggcagaggaattcttgttactcatttattaggtagtgaacagaaatgaccatagtcaacatttgcaggcaggtggaaagttcagaataggtcttcaggttgttggcctgatagtgtagtgcaaggccagtatacaaatggccactgagtgaagactctcctccttccaagttcagcctcatatcctacctttctcttcactgcagcttcagctaacatcttccttccatttgctcatttattcacttagtattgcaatcaacatcgtctctcagggaagaaataacttaagacttgaacttcgagtttactttttagtggacaagtacagaactatggccagtagtgccaaaagaacgtggaatgcagtctccaaggtcagttccctctaatctgtaccccagtgatctgccctgtgtacctgttttaaccacaatcagtttgctggaaactgaagaaggacactgatcataggataggtcaggttttagaagcactatctgataaccccgaagggacaatatgtgtaataaaactaggagaaactatgaaaacagaaaagcctcaggagacagaaaaggcggaattattccttttccctggaaatgaaatctcatggccttttaaacacagtgcttaattttcccctgtgatttttagttatgttttgagaagtaccattttccttctccttcacatatgttagacagtaagaactggcagtgctgggatggtaagactgatgggttttccacatacccaacaaaaacccatttccatcaagggctacactatagcagctgagagcttcataaaaatttttcagcattgtgtgctgggcacttccagttctgtgatctcatgaaagtcaaccaaccaggtctaaagacagagactgcttccacagagaacaggaccacagaagggtaccactctttggagatgctgccaggaagttaaagaaacctccaactctttttttaaaaattttttatttttaaatcttctacctccaacctgctggctctctctgtactaccactctagaagacaggatgggatagaagaactgtgtgtattaggtctgtctctctacaaccccagagactgagtagcctgcttggagatagatccgtgattagaggaaattttcccttgtcttctttttctcaagtgtgtatttctttgctccagattcccatcttcctctctactttgaatattaagagctaagcttaggtgattttgtactactaaaacaataaagatgtacaactcaatatccagtttaaattgaagaaaaatacaacaagactaacttactgttttgctggacacaaaatccatagaaaacttgtcattgtaacactgagggagagacagctttatctatgcaaaccactgacaaatattgtgaggtgaacactgctgaaaagcgaggccccaaggtagaacaaaaagagcactgaacttgtaatcaagattatctgtctctgagcttgtaatttactacctatgtcctttagcaaatttcaaactccctgtgcctcagctccttcatctgtgaaatggagataattatactggtccttacccacttcacaaggttagcataataacaagaaaaaaaaaaagggatcacttgcgaaagtagtttgtagactgtgaagcactatgagcggtagaatgggatcacattcgcttcactaaaggaaaaccccaaattccgatagctgacttattcctccaacagaatacaaccatccctgaatactggtaacagttaaaaaaactgctcagcagggcgcggtggctcatgcctgtaatcccagcactttgggagaccaaggtgggcggatcacgaggtcaggagttcgagaccagcctggctaacatggtgaaatcccgtctctactaaaaatacaaaaattagctgggtgttgtggtgcacacctgtaatcccagctaccagggaggctgaggcaggagaatgacttgaacccaggaggtggagattgcagtgagccgagatggtgctactgcactccagcctggatgtcagagcaagactccatctcaaaaaaacaaaacaaaacaaaactgcttacagcttccagatgagatgaagaaaaggtgcagtaatgaggagtgatgaccatcagcttgcagcactgcgatacactttctgtttcatatagagagacaatgacattctctacctcccaactattcctaggagaattaagctgctccaaccatgaccatataggcatgatttcaccaactagtgccagcctttctacttctgtattggttccagctcggtatccctaactgcctaacaggtatttccacttggatgtccacaagctcaatttatttatgtcaaaaaaaatcatctttcccacccacattattttcctgactctattcctgtcctctgtatcattttcccctgtcagttttattgaggtataattgacaaataaaaattgtatatatttaagttgtacattgtgatgttttgatacattatgaaatgattatccaatcaagctaattaacatgtccatggcctcagttatctttttttggtgtagtgagaatacttaagatctactctccaagcaaatttcaagtatataaaatattaactatagtcaccatgctgtacattaggtctccaaaacctgttcatcttataactgcaagtttgtgccctttgaccatcatctcctcatttttcccatcctctgacccctggtagccatcctctactctctttttctatgagatccacttttctgagattccacacactggataaacgagatcatgcagtatttgtctttctatgcctggcttatttcacttagtataatgtcttccaggttcatccatgtggttgcaaatagcagaacttcaagaaggctgaataatattctgtcgtgtgtatgtaggtatataaacacacatatcacattttctttatccattcatccactgacaatctgattccatatcgtggctattgcaaataatgctgtgatgaacatgggcatgcagatacctctttgagataccaatttcattttctttggatatatatccagaagtggggctgctggatcatatggtagttctatttttaaattttttgaggaacctctatactgttctccacaatggctgtaccaatttacatcccactaatgatgtataagggttcccttttttccacctcctcaccaacacttgttatcgtttgactttttgagaatagccatcctaccaggcgtgaggtggtatctcattgtgttttgtttttttttgtttttgttttttgagatggagtttcactcttgtccctcagggtggagtgcaatggtgtgatctcggctcactggttcaagagagtttcctccctcagcctcccaaggtagctgagattacaggtgcacaccaccacatctggctaatttttgtatttttagtagagacgggattttattacgttggccaggctggtctgaaactcctgacctcaggtgatccacccaccttggcttcccaaagtgtgcccggctcattgtggttttgatttgcatttccctgatgactgtgatgttgagcacctttttcatatacctgctgggtgtttgttgggtgtttgtatgtctcctttggaaaaatgtctattcaggtcctttgtccattttttatttgggttatttgggtttttttttttttttttttgctattgagttgtatgagttccttatatattttggatattaatgccttactgaaaacatggtttgcaaatattttctcccattctgtaggctgccttttcattttgtagattgttttctttgctgtgcgttatcaccttcctcttagctatctgtattcaaatcttggtactactgactccgtcttatgcctcactgttagtcttcaaagtggaaacctcttgattccttcttcattgcatttgtcaaattcatttttcacttgccatttacattgtcaccattcatgcttaaactactataacagtctttcttctttcctttttctgtaatctgtagtagacacaacaggcaatactaccttcctgtggtttacagtactcatatcattctcatactcaaattttcaataagtccatacagcttccacaataaaggctaaactgtgctagcatttaagctaccatcagacagatttctcaagcccaaatctaatattactctacttaaaatacctccacgggccaggcacaatggctcacgcctgtaatcccagcacttcgggaggctgaggcaagcggatcacttgaggtcaggagttcgaggccagccggaccaacatggtgaaacccaatctctactaaaaatacaaaaaaaaaaaaaaaaattagctggtcatggtggtatgcgcctgtaatcccagctactgaggaggctgaggcatgagaatcaaatcgcttgtaccctggaggtagaggttgcagtgagctgagatggcgccactgcactccagcctgggagacagagtgagactccgtctcaataaaaaataaataaaatccctccatgaactggggaaaatatttgcaatatgtgtgacaaaaggttaatgttcataatataaaaagaactttttaaaagtcacaagaaaaagacaaaatgaaaacagacataggacacaaataggtgattcatacaataaaaatgactaatacatttaaaaatatgatcacttgtaacaaaaaacaaattaaaaacattttctagcatgcacactggaggattagaaaaggtaaattattttaagaaaatttaaaaaatatttcatttcttagattggtaaaagttgaaaacagtcttgttaaggatatggggaaaatggcctctcagaccctactggtgggagtttatttcaaagtgcatatactctgacccatttctaggagttcctaaagaagtttcacataaatttataaatatgtaaatatgttagtttgtagcaccgtttgtaatagaggaaaaaggaatacctcaaatacccatcaatagataaaggccaggcacagtggctcacgcctgtaatcccagcacttcaggaggccgaggcgggtggatcacctgagttcaggagttcaagatcagcctggccaacacagtgaaacctcgtctctactaaaaatacaaaaaattagccgggcttctggtggcaggtgcctgtaatcccagctactgcagaggctgaggcagaattgcttgaacctgggaggcagaagttgcagtgagctgagatcatgcgactgcactccaacctgagcgacagagcgagactccgtctcaaaaaaaaaaaaatagcttggcaacataaattattaatatatccatatagtcctatgcaacaatgaaaaggaatgagctggaactgtatgttcttagatgggaacatagccaagatacattaaaaagaaaaaagcaaactacagaaagccaagtatgagcctgtttattttatttatttatttttttaaggggaatggttcatagctaataccgtatatgtagagaaaaacctgaaaggatactcaaactcttaatcaagttatccttcagtgatgaaattagaggaaaattctcttatttatttgtttgtttggagatagagtcttgctttgttgcccatgctggagtgcagtggcacgatcttggctcactgcaacctctgccttctgggttcaagcaattctcttgcctcagcctcctgagtagctgggactacaggcttgtgccaccacacccagctgatttttgtatttttagtagagatggggtttcaccatgttggccaggatggtcttgatctcttgaccttgtgatccacccgccttggcctcccaaagtgctgggattacaggcatgaaccaccgcacccggctttttatttttattttttgagacagagtcttgcactgttgcccaggctggagtgcagtggcatgatcttggctcactgcaacctccacctcctggattcaagcaactctcttgcctcagcctccttagtagctgggattacaggcatgcactaccacacctggctaatttttgtatttttagtagagatggggttttgccatgttggccagcctggtcttgaactccggacctcaagtgagccacccgcctcgacctcccaaagttctgggattacaggtgtgagtcactatgcctggttcctttttaaaaatgtctataatttgaattttaaaaaacagtgtttattcttggccctactaccaactagctgtgtgaccttgggcaagttccttaacctttctactactcagttttcccatctttggtaggtacaataatgactcccccaaaatgtccatgtcctaattcctggaatctgtgaatacgtgagcagcgagtaacgttgctaatcagctgatcttgaggtgggataattaacctcgattgtcccagtgggcctaaggtaatcacaagggtccttaaacgtggaagaggaaccaggcatggtggctcatgcctgtaatcttagcactttgggaggtcgaggcaggtggattgcttgaggccagaagttcgacaccagcctggccaaatggcaaaaccctgtctactaaaaacacaaacattagctgggcgtggtgacgcatgcctgtaatcccagctactcaggagactgaggcatgagaatcccttcaacccgggaggcagaggttgcagtgagctgaaatagtgccactgcactccaacctgggcgacagagcaaggctgtttcctgcatcgcccctcccgcaaaaaaaaaaaaaaccaataaaaacaaaaaaaatgacagtggaagaggaacagacagacgtggtggctcatgcctgtaatcccagcattttgggaggctgagacaggaggatagtttgagcccaggagtttgagacccacctgggcaacatagcatcctctgccttggtccccctaagtgcctatctctataaaaaattaggaaaaaaaaattagccatgtgtgttggtgtgggcctgtgatcctagctactaaggacactgaggtgggaggattgcttgagcttgggaagtccaggctgcagcgagctgtggtcgtgccactgcattccatcctgagcaacagactaagaccctgtctcaaaaacaaaataaaacaaacaaacaaacaaacaagtggaagtgggaggcagaaaaggtcagagtgatgagatatgggaaaggtttcatcagctatagctggcttttgaagatgaagaaagggaaccatgagccaaggaatgtgggcagcctctagaagccagaaaaagcaagaaaaatgattcttccctaaaatagctgctagagaggaatgcagctctgccaacaccagttttacccgagagagacccattttggacttctgacctctagagctgtaagataattaatttgtgttgttttaagccacttataaaagaagtaatgtttatgtttttcaataagaaaaaaaaagattaaaaatgccctttcaatagttctctacaacagggtgaaatccaggccagatgtggtggctcacacttgtaatctcagtactttgggaggccaaggttagaggatcacctgaagccaggagttcgaggctgcactgagctatgaccacattactgcaccctagcctgggtaacagagcaagtccctgactcttaaaaaaaaaaaaaaaaaatggagcctaaacacttcagcatggcatacagactctcattaatttgacccaaactccaatctcattttctcacctctacctttgctatgatctgtatgttttgtgtccttccaaaattcatttctgttttttctgaggcagggtcttgctctgttgcccaggctggagtgtagtggtgcaatcatagcgcactgcagcctcaaactcctaggctcaagccatcctctgtcttggcctcccaaagtgctgggattacaggcgtgagccaccatacctggccctgtttttgtatttttttgtagagatagggtctcactttgttgcccaggctggtctcaaactcctagcttcaggcaatcctcccacctcggccacccagggtgctgggattagaagtgtgagtcattatgcccagcctaaaaattcatatgttaaaatctatttcccagccaagcatggtggctcatgcatgtaatccccacactttgggaggccgaggtgggtgaatcacttgaggtcaagcgtttgagactagcctagccaacatagtgaaactctgtctctcctaaaaatacaaaaattagccaggcatggtggtgcgtgcctgtaatcccagctactcaggaggctgaggcaggagaatcgcttgaacctgggagacggaggttgcagtgagccaagattgcaccactacactccagcctgggcaataagagtgaaactccatctcaaaaaaaaaaaaaaaaaaatctatttcccaatgtgttggtagtaggagatggggcctttgggaggtgactaggtcatgaaggtggcagtctcctgactgggattactgcctttatgaaagacggcacggggaacttgttttgccccttctgccatgtgaggaagcagcaagaaggtgccacttatgaagaggagggccctcaccagacaccaaatttgctggcaccttgatcttggacatccagcctccagaattgtgagcaatacatttccgttgtttatagattacccaaatctaaggcattttgttatagcagcctaaacatagagaacgctacagtcctcctgccagctccagctataatgaatatccactattctccaaatttcctgtaatcttccatttggcaagcttttacccagcttgagcaccctctcctttacaaggatttccttgacctcatcctcgccctccatcactacaagaagtaaagacttggcgctctctgcactgagacacaattctttttacatgtccacctgctttctggactgcccttcctagacaggaacgttcttttccccagccctgcatcctacatacctaatgaagtacctggcacatggtaggtacatcactattgcttatattaatgacctaaacaatctgccaataatctaagcttatttcccaccgctctaaacataaaccctggattctactggctccttcccaaacctgcataagaattccaaacttcttttgccccaacctgaaattctatctcacctcttgatttttatccatcttaaatgctacttcaaaaactctttcttgacctccttcttctttggacttcagtggcataggcctttatatcccctacaactcctactgtaatcatggacacataaaaggtgtgtaataaaaaatactctgtttaggctaggtgcagtggctcatgtctgtaatcccaacattttgggatgctgaagtgagaagattgtttgaggctaggggtttgagaccagcatgggcaacatagcaagcccctgtcactactaaaaaaaaaaaaaaaaaatttttgtttaaatatgaatacaattatgtgaaaaaatatttgcataaaagttgattgaaggcaaatttatgaaatgtaaatagaggttttgtttgggttgctgggccctaggaggtttggattttcctttcttccgccccctcccccgcctccccacccagatggagtttcactcttgttgcccaggctggagtgcaatggtgcaatctggctcattgcaacctccgcctcccaggttcaagcaattctcctgcctcagcctcctgagtagctgggattacaggcctgtgccaccatgcccggctaattttgtattttcagtagagatggggtttctcgatgttggttgggctggtctcgaactcctgacctcaggtaatccgcccgccttggcctcccaaagtgctgggattacaggcgtgagccactgtacccggcccattttatttaacgagtaggtttttcatctttcattataaaagtattggaaaatttgtataccctttaatacattactgtttccaccatattgaaaacttgttaaatggaaaaacttcaaggaggcactgtagtagagtaaagggcccagtttctggagcaacaccacttaaggttaaaaaaaaaaaaatcacagtttgccacttgctagctgtttcatctttgagcaaagtctaaattttttgttcctcagtttcctcacatatttatctcatagggtcattgtgaaaataaaaataatccatgtgaagtacttaggtgagtacttggtttataccaaacactccgattaacattagctattggccacaacagttgaagctggaatggctgtcaaaaatctctgcacttgcaaacaaaaagctgatattcaaaattaaatgacagtcactaaggtgacatatcttagtaagtggaacttgtcaattaaacagcttgggatatgtctgcactgcatgctattctaactgcacctaatttggccccaaatttaattacatgcatgtctctatttcacacatgaacatgttctcaaaagatatctaacacaaaccaagagtttcaaaacccaaagggctcagttctgtttctctaaatgtctgggcttattttctaaaataggtttttcaggccaaatgtttcccagaaacctaaatgacagaatggagacagagaatgagaagacttgcagttatgccttggctgtattacaaattcaaccagctgcctttcagtcaaatttcaagacatttgttccctgaaacacagaatgggaagaattgcttactttcttatttcaaagatagtgtaagaggcatatacaactcacagatctgagggacgaattctatacaaaataaatcataaaatacctctttcctcttcctatctgctttctttattcccactaacatatagttcttaatcagatgaactttaacttgattgcaaattaaattagactataaaaaaaaggaatcaaaacagtacccatcatgatgtgatggttaattttatgtgtcaacttgactggaccacagggcgcccaaatacttggccaagacattattttgggtgtttctgtgagggtgttttggatgagattaacatttaaattggcagactgagtaaagcggattgttcttcccaatgtaggtgggcctcatccaatcagttgaaggcctcagtagaacaaaatactaccttcccccaagtaaaagagaattctccttcctgacaggctttaaactggaacattgacttttccagcccactagacaacagctctgcagattttttttttttttgagacagtgtctcactctgttacccaggctggagtgcagtggcatgattttggctcactgcaacctccgcctcccacgttcaagtgattctcctgcctcagcctgccgagtagctgggactacaggcgcccaccaccatgcctggctaatttttgtattttctagtagagatggggtttcatcatgttggccaggcttatcttgaactcccaacctcaaaggatccgctcgcctcagcctcccaaagtgttgggactacaggcgtgagccactgcacccagccaagctctgcagattttggatttgccagcctccataattgtgtaagccaattccttataataaatacacatatatttatatatctatatctccctatatgtttatttctatatatcttttacttataatatttaccaatctctcttattggttctgtttccctggagaactctaatatagaacaataaataccattataccaaaactgcagctaaaacttcagagaattcaggtcatgctggaaaactaaaggcaggcagggtttttctaacaacaaaggtcatatattctgactatatcctgaagtctctggtatttatggcagaataaaaaaatatgtagaaatatggtgaaaccctgtctctacaaaaagtacaaaaatcagctgggcgtgggggcatgagcctgtagtcccagctactcatgaggccgaggtgggaaggttggaggattgattgagtctaggaggttgaggctgtagcaagccgagatcgcaccactacactccagcctgcgtgacagagtgagaccctatctcaaaaaaaaaaaaaaaaaaaaaaaaagacataatgcaaggctgggtgtgcggtggctcatgcctcctataatcccagcactgtgggaggtagaggcaggcagatcacctgagctcaggagttcaagaccagcctgggcaacatggtgaaaccctgtctttataaaaatacaaaaattggccaggtgtggtggcatgcgtgtatagtcccagctactcgaggctgaggtgggaggatggcttgcatccagaaggtcaaggctgcagtaagctgagattgtgccactggactgcagtccagcttcagtgatagagtgagaccctgtctcaaaacaaacaaacaaaacccaactctctctatatataatatatcatatatataattatatgtagaattctttccagaatacctcattttctagtgacttcctgcctattctaacctgcagctttgggggttatttggctttaacagatgagtcacttacacagctgaggaaatcttcctatacacagtgaaccaagaagggtggaggggaaggctgggtgcagtggctcatgcctgtaatcccagcacttcgggaggctgaggcaggtggatcacgaggtcaaagatcgagaccatcctgtcccacatggtgaaaccatgtctctactgaaaatacaaaaattagctgggtgtggcggcaggcgcctgtagtcccagctactcggcaggctgaggcaggagaatcggttgaacgtgggaggcggaggttgcagtgagctgagatcgcaccactgtactccagcctggtgacagagcgagactccatctcaaacaaacaaacaaacaaacaaacaaacaaaaaggttgaaggggaaaagtacattgagtttagtttccttgggcaatctggttactagattttacagaattccatggaaatttttacatcctctaaccatggccttagccactgcctacaaaagtatcaggcaagacaggcctcacgttagatgagatagtatcctgaggaccgaagagagaccacctacagaaaaagttaaatctggagataacaggaaacagtgagggaccctacctggagaaagtgaattagggaaacaccttggggtaattctggcgcaatagtagtgataaagcagcagaccattctttactgctaaagggccttccctgacctacaatctcctctgctccacttatttggtcactcagctaagtgaccaaatttcttctgttcaaagaagaaagtcagggcagacactaccccacagctgtgttctcagccctcccttagggtttctgagaacactctgggggaactgttttcttttttgaccaaaagccacctgagtggttggagaggcatcttgtctcaaatgtaggacctcctctagggaggggctacgatatctacgttccaaacaattttggacgctacctcttttgaatgcaccaaagaggtagcatccgagtgataagacctaattatttttagtagcatcgcatttccattcatgtaaatattttatttttcctaatcataattgcttttctcttatggataggggcacgaagaggaattaggtatatttcagttccttctttaattagtttcaggcctataatgttcaccagttgggagagaatatccagaagggctggctggctggccagcctctaacaatgcttgaaaaggcaggtaaatcctgagtcagcaaatgggaaaagcaagcacattcagtttttcaaaaaggtcacgtttccaagtagtatttggcatgttccatcaagtactgaattggtactaggcagatggatctaagcaattggtattagtaagttaacaggtaaacagaataatatttaccttcattttaaaagaaggtatttaaccacatttctcacttgtaagtgggaggtaaacattgggcacacacataaagatgggaacaacagacactggagactcccaaaagtggggagagagggagtaagcgttgaaaaagtgccgactgggtgctatgttcactacttgggagacaggctaagcagaaacccaagctttagcatcacacaatatatccatgtaacaaacttgcacacgtaccccttgaattgaaaatttagaaaaaggtatttaaaaaataaagtctccatttccgcaatcctcttgagctatcagtataaaacagcactttgacaaactcacattaaaggccaataaccaccatgaatacaagacttagttctcatttatttgtgattttgcaggtgttcaaaccaatgaatgaaaatcaattatctcttcatatcaatgaaattcactatttcactattatcttcagaatcatagtgatcaaaaccctacctgaaaatggtaatacaaaagagaactattaatacaaggtttcagaagactgtgcaagttaaaataattggcattaaaacgacacacaacaaaccaccgaaggtttggtcccttttctctctgatatgtggcctctgatctctttcttagggcagtggttttcaacgtctgtgtagcagaatcacctgaaaagctaacagaatatatagaaacccaggatttgtatttgtatttaaatgtaaatacaaaaggtctgggtctctgtatctttacaaagttctccagcaatggtttccaaaccaggcttatcacaatcaccagggaagctctgaaaacaacaacacattcctaggcttcatccctagaaattctgattcagtaggtttgaggtcgggacccaaaaatctttttctttttgttttttttttttggagatggagtttcactcttgttgcccaggctgaagcgcaatggtgtgatctcagctcactgcaacctctaactcccaggttcaagcgattctcctgcctcagtctcccaagtagctgggattacaggtgcccgccaccacgcccagctaatttttcttatttttagtagagacggggtttcagtatgttggccaggttgatcttgaactcctgacctcaggcgatccacctgcctcagcctcccaaagtgctgggattacaggtgtgagccaccacggctggctcaggacccaaaaatcttaaaacatttttaaaaaattttaacaaacttcccaggtattcccgaccagccagatttgggaaccactgacttaggacacttatttaaggtctatcacagaacttcaggcctcagagtttagtaagaatatcgataactttgggtaggttataaatcaccatcctagagataatttaacaaattaaatggtctagtagtgatttgatactaaaaagccctgcccaatttagtacttaaattacctaatgattttctgtctatctactttcctcccccaggctaggacctgcacataatatgtttcctatgactaagtgcctacgtgttcacaaagttgccccagtggaggttgttaacttctctcttttcttcttccattcagattcccaaagctgtgaggagcagacctatttcgaagcatcacagccagctgatgtcacttgcagtattatgcattaagacatcaacccagaaacctgcaaatgggagacactaggcaatcctatcatgaggattaagctctttgtggaagaaaatgctttcattgcatgagataggtagtttaaaaatgactattcttttttcttttttttttgagacggagtccttctctgtcacccaggctgaagtgcggtggcatgatctcggttcactgcaacctctgcctcccagtctcaagcgattctcccacctcagtctccagagtagctgggattacagacacgtgccatcacgcctggctaatttttgtacttttagtagagacggggttttgccatgctgaccaggttggtctcgaattcctggcctcatgtgatccgcctgccttggcctccccaagtgctgggattacaggcatgagccaccatgcccggccaaaaaacttgactattcttgatgccaagacaagagaaacttaattatgacgttagaagtttcaaaaatacagtgacttctgggacacttctagtagccaaaaatccacagatgcccagaccccctccttctgcattccagaatcagatgtttacattccaagacagaaagaatctgaaacaacggcctacaagaaatttgggaaatgacatttgatctcattttcctctcaattggaagtcatgatatcaatgaatatcaaatggaaaaataagctcagaagtaggtgagaattatgatctctaaaacgcaggtgctgatttctaatccttctcataaaattccggatcacaaattgagggctgatgagaagatcttacaccgaaggcactaactggcactaatgtgagccagcaacatgtgaaaggctaatccaggagatgcagaaatgcacatgggttccaggtgtcttttctaagtgacaatgggcctccttactggacagtagtcaggagacaattcaaatgtacttaataaaattgtcaggtgggcaaccaaagggaagagacttaaaagacctcccagaactgggatggaaaataagccaaacactactagcagcaggaccagctggaggacttggtttgtagattgatgtagtccccttgggtggacaaagacatgatatcttctgtggaatttctcatcatcttttcaatgaggactctaaaagacaaaaaataagcctgagaagcttattttggaggaaaagcagaaatggcagatgtagtctgacttatcatcagagagtatttggtaaagccagaaggtttaaatgcccctttgtccccagttatctcaggaaagacagtatccctgacctttaggggctagcattccaatggctcagtctgtcattgttggctcagaaataagaaaagagggtccacagggccacagtggaagatggatacatctgcatgcctatcagcatgagctacttacctcatagcctcattaatatttttgttctccttgactgatgtttctgtccaacctgtgaaaccgttctctttactgaaccggtcaatctggtcccggctcactgcccaaggggacagatcacactagcaaagagaaaaaataaaaggcagtatcataaacttcctgcaactaagaaagaatatggctcagatactgtggattttaaacatatttccaccaatggataagaacaccagcatcggaaatctataatcaacattcttcccaaagaaagtctcacccttggctgggcgcagtggctcacgcctgtaatcccagcactttgggaggctgaggcgggcagatcatgaggtcaggagagcgagaccatcctggctaacacaatgaaacccagtctctactaaaaatacaaaaaaattagctgggtgtggtggtgggcacctgtagtcccagctactcgggaggctgaggcaagagaatggcgtgaacctgggaggcagagctggcagtgagccgagatcgcgccactgcactccagcctgagcaacagagcgagactccgtctcaaaaaaaaaaaaaagaaagaaagtctcactcaccctcaacatcctttgaaggaggtagagatgattttgccaacttaagaaggggaaatggatgcccagaatcagagagcattttacttcctttctaaccacagatagaggctagggaccattttctgagattggccacataccttgttggccaagagcaggcagggcaccggctctccattgggtagtgtgagcttgctgtctaggtcctgtttccacctctggctgttgctgaaggtagtggcattggtaacgtcaaacataataacacaggcagaggcatcccgataatacaatcgtgtcatagaggtgaagcgctcctgccctggggagaaaggggagagttctcaaggtgacccaagagccggcctctccccattccttgtagaagagggcagtaagcatatgtgtcagatggggccactcactttccccctctgactcttggttttctatcccataaagggataatgaagcccaattatttccaaggcagattccgcacccagattgctccagtccaaatccctgctctgctgcatactatttgacttcgggcaaatcaagctctcagtgcttcagatttctcatttgtaaagtgaagataaaagcagtcgctttttttttttttttttgaaacagtttcctgcactcctgttgcccaggctggagtgcagtggtgccatctaggctcactgcaacctccacctcccaggttcaagcaattctccaaaagcagtagcttttatgatagggttgatgtgaggattaatgagtcagtgaatttaaaatacttagaagaatgcttggcacatagtaaggattcactatttttactgtatctattttctggggatcttgtttttcaccaaggtcagccttaaacctagaaaaagcaccctcccctgctgtgggagtgtccacctatagtctggacaatccaccaccttgccagcccctccatccacatagagactgctccagatctattcagggcaaaacatctacaaaagctctgcacctattcagctcatgtgtcctcagagcagctcaatcattccagcttcagaaaaacaatttctggctttgctgccccattttttcctcagagctttctagttaaatcaaaatttcttcccttgttcctatctagccctcccactttacctgcaatatcccacagctgaagccgcactatctcgtagtcagaccactggagaaccttcagagcaaaatccactgaaaatatatgtacattatactttaataaaatttcactgtaaaaaattaatagggataaactcaaatcaaataggcagtgaaaccctatggacacacaactccaatcccatatgtttaactttaagccctcaattcactgagatgagtccacatgcgtgtatttagtgtgagatggatgattcatactcactctccaaaggggtttccagcttttactctactgtcaagctcatttatttgctactgtttgtctccaagactgggggtgggagtaactatgaaaacaattctcattctcaggttaaatagtttctgggagatttagggggttttctcagggaaggggtgatgggggagaagggggaaatgagacaagtgtggttgctttcgtatcttccacattcaatttcactgttggtttctaatcaaattgtattatgaaaagaacacaccctggggaactctacatccaccataaggttgcaggtattatcttgggcaagaatggaataaatggaaaaggtcccagaggagtcccaagaagaagacactgtgtggatgttgctgaagagtcctgctggaatctaccaccaagtctgcaggtgctgagactccttaaggctgagtaagtattccatggggaaagccttttggctaaggagagaaacagagtaatttctgaggtttggaaatattatctttcacatctgtgacaggaatcaaagctaagggaaatttagactaaacactgaaaaaaaaattagccaattatattctttgctaaaggaaaactacagcaattgttaaaaattaactattaatagcaggccacttttaacccaaatccgtgaaatagggacccttatattatttaggagtgggagggcagagcggtcaggatagagtgtctgaaactttgaacctttaattttgccagacttaaattttttgttcctttgtttttgagacagggtctcactctgttgcccaggctacagtgcagtgagtggtgcgaacggggctcactgaagcctcgacctccccagttcaagcaatcctctcgtctcagtttcccgagtagctgggaccacggctactttcttctttaatttttgtagaggtgggggtcttgccatgtttcccatggctggtctcgaactcctgggctcaagcaatcctcccgcctcagcctcctaaagtgctgggattgcaagtatgaaccacggtactgggccctactgggggttcttaaggagaatgttttaattgcaatgtaaatgtttgttaatttctttttaaacttccatatgaacaggagcacacattttcaatttttccattggtacgagttttccccccttgaaacaagttcttttaacagagagaaataaaattttaagttactctcccccatcaccagctcttcctagctaaataccttctaattaacaataaggcatttctgcctctgaaaaaatagttgagtccaaaggccacacccgggaaagaaatgaatgaactcggtgtccccttcctccctaccttctccagtttgaggaaaaaagtggtgggaagataggtcagagaagtggtatatttcacattcttggaagaattccttggttacctttatttaagcaatcaacggacaaaaacacagctcatcagccctcatgggcatctgactgcgtagccaaggggctcgttcggggattttgtgtcttccatcccacccacagccccacaacaaagctacagtccttcagaccagttccgcttcctgcgttctcccactgaagccaggttaaacaccttgcggttcctccctcaacagaggggcaggactacagccccagccggcacctaaccaggaggccccacagaggatctcagctgcttctgctgattggagagatttgccggacagctgaaaggctggagacttaagttcacagtacgcctgcaataaacagcaattgctcatcctcatcctcccttccctatttctcatcttcacgcctttgctcttacctttctcctggcagtgggctcagtttgggaaaatctaacgggaaactcaagagaggcgtgtaaaccaaacacccggcaattacaccatctaggttcccagacagtacttcctgacccgaagaaggacccaacaaccgacagcaaatccccaccccacttgggtccccagctcgagtccgcggtcggggcctcctcctccccctccccctccccacccccgagacgtctcacctcccaccgtggacttgtagtgtttgctgaagctgtcctgggaatatcgctgcaccagcgacgtcttgcccactgcggcgtcccccaccaccagcactttgaacaggtggtcgcggctgcccatggctagcggggtgtgcgttttagggaggcgggaagtgtggtcggggatcgggggtcgctcgttttaacccctttggatccggaccctcttcaaactgaagtgaggcattcccacccaccgcctgtctgggctgctctgacgagaaagcaaaaaaggaaactttgcactcaacctatacgcgcttcctccccgggcggccgcaacctgggtggggcgcagggcgcgagctccgagcccccggctgttcgcaccttccccaccccctcctggcctgactgccgagaaactggaccaggcgccgcggaacctcacccaccgggacttcccccgagcggctccaagtcagtgactgaatcccagtcagctccttacaccactggggccagatgatggggaccctccccttgcagcacaaaccaaattgtgaggaaggagcagccggcacctcgattccctagacgccctcccgcgcgcctctctctccccttcctccgcaagcgtcacgtgcagggttgcctgtggcactacatttcccagctttcctcgcggtaaagagaaccagccgagtgcggaggctcaccgcgaagcctcctgggaaatgtagtatattcgttattttgttttaagcaaacctacaccaagtttcaaggcttcaaactccctcgacagtttggaatcttattttgaaacaattctaggtcagtaaagatcccttaaggggagatttgtgcaacgtgatctcactggcctgaatccatccccagatagttttctcctgtctttaaaggtttaactgagttaagattgaaacttatttcattagtaaaagcccaagcctcatccatcatgctccaagtgaagtccatttcctattccttcaagtagatagacaagcccaggactttgtgaaatgactcatattttctgtgtgaacttgcccaataccaggcaagttcaggaaaacttgacccaagagaccagtctttggaaaaaaacctatgccaaaaattacagcatttaatatccagcaataacaataaagatggacagaaaacaagagacagttctccattcatacttctacaatgcctattctagccatactactcatgtatcacttgagctagaagctaattgaaatacactgggactccttcttgatttgttgtggctgttgttaatagataatcataaaactagtgtttggcaaataattttaatttctcagcctgtaactttactgacctacctgtcacttgggtagaagttggcaggacatgagctcaatggcaagcaaagagagctccattttctatacttttctaggaatagaggaagagaaccagcggggccatgggaaaacagcccaggaccagacactaggaaatctaggtctcttgatagagaggctatcacttatgttttgtggcgaaagaacatcagcatggttcacaatatattttgcccagaatgttcgttacccaggtacaggaggttagttcaagctactcatctttaaggatccagttttctctgttcttattcgttttgacatagttgaccactccttgacatttgtttcccttatgccttctatgacgctgttctttctttgtcatccccgtacttctctgatgattatctttttctttcaggtttctctccatcccatttcccgctaagtatttcctaaggcctgattcttggtctctgagtcaatcattcgataaactctttagtgaattgtccttggtgtcaaagatctatcttcactttatttgttctttatctctgatcagtgatattctgtcaagaccagctctgttggggagaccctaacccagtggcgctagaggaattaaagacacacacacagaaatatagaggtgtgaagtgggaaatcaggggtctgatttcctttagagcttttagagctgagagccccgaacagagatttacccacgtatttattaacagcaaaccagtcattagcattgtttctatagatattaaattaactaaaagtatcccttatgggaaacgaagggatgggccgaattaaaggaataggttgggctagttaactgcagcaggagcatgtccttaaggcacagatcactcatgctattgtttgtggcttaagaatgcctttaagcggttttccaccctgggcgggccaggtgttccttgccctcgttcctgtaaacttacaaccttccagcgtggacgttagggccattatgaacatgttacagtgctgcagagattttgtttatggccagttttggggccagtttatggccagattttggggggcctgctctcaacatgtccctcttctctgatttgcaaattgataaatgcaaaggcagctttgtcacggtgagctacttctcgcaggagtcaggatacacatctgcagactatacaaagacaaacaacacagattaaaagcacaatcatcattgaaatcacagagcttccaagtgtttttatccattttcggctcctttaagcactccagttcctggcattaaggtcaagtgtgcctcggatgctttaaatatttcttcttttaattttaaatccttatgttaagctcctagagcgggccatatcatttgaggttgaggtgtcactatactgccatggttccagataataggaactcttgctgtacttcttattatatctaccatctgaccattttgttcagaccagctgaacatagtgtggccgtggcacgcagactgagaggtgcaattcaagctaaacatccccttaggggaccaattaataatgattccataggaatcattgtgcagcatctctgcctgttctgcaatgcaatcttcctaaacaagtacgttcattttttctaactgggtccaatcctgtttacaaataagtttttgagggcggtatgcctcaattataggagcagatttattatggtaaatactgagatcagaaagcatgtgtaactgcgtcataaagtgattgcatccaggcattattgccagccaagattgataaatatacccaataagtataattgttctctgtgtcagcccttaatgaaggaatactcacggcactggtgataaccgctatcatagctaccattaacactttatttgttctttatctctgatcagtgatattcagctgcccaaaaggtgcccccacttggatgtcctgccacatccttcctcttactacattgccataaaaatagctccttttctcagcttccctatttctgtcactggtctcatcatttcttgcctccatgtagacttcagattctgagcattattatttcctttacacatgtccctttatacctatttatttgtttgtttgtttattgagatggagtctcactctgttgtccaggctggagtgcattggcatgatcttggctcagtgcatcctctgcttcctgggctcaagtaactcttgtgcctcagcctcctgcgtagctgggactacaggcgcataccaccaagcctggctaatttttgtattttttttgtagagacagggttttaccatgttggccaggctggtcttgaactcctgacctcaagtgatctacccgcctcagcctcccaaagtgctgggattacaggcgtgagccgccgcacctggtctatacccttttaaaaaaaattcagttaccatgtctgattgattgtttcttcagtaaatggtttctcccactcatcctctctgcttcatattcagtaatactttccttttttttttttctccaacttttattttaggttcaaggggtacatgtgcaggtttgttacacgagtaaactgcatgttgcgcgagtttggcttacagataattttgtcacccaggtaatcagcaagtaacactttcctagttcaggctttcaccatctcacacctggattcctgcagtaacctgtttattggtctccctgaatttattttctttttaactcaccgtctacaactggacaggatggttttcctaaaacaccattgtttgttcttccttgtctaccaactgtctttcaaaaaaaaaggccaacctccctgaagctggtgtccaaagctttctatgcacctgccccggcctacctaaccaattttatctcacccgacttcaaatgggagtttccttcttccaacaaggtgaggttccttatgctcttttaaagcccaatgtcatttttgattttctgtttttgtccaggatgcatcacctttcagaatactcttcaggtttctttctacacatctaaatcttacttaaatattattaagaaaatcaaaaggaagagaaactatattattcactaagtgggagtggattgtcttaaaggtcaccgaaggttctaaaattttagtgtgcataagcatcacctacctggggtacttgttaaatacccacattttgattctgtagggctagggggtgacccaggttaatctgcatttttgacaagtactcatgtgattgctacaccacattccactttgagaaatagtacttttgagaaatggtgcttcaaggcctgacttaaatatctacttatttataaacatttcccttattattgcagcctttattggtcacctgtagcatttatttttttattttaattttttaattttttttttttttttgagacagagtctcgctctgtcacccaggctggagtgcagtggtgcgatctgggctcactgcaagctccgcctcccgggttcacgccattctcctgcctcagcctcccgagtagctgggactacaggcgcccgccaccacgcccggctaattttttttttttgtattttttagtagagacagggtttcactgtgttagccaggatggtcttgatctcctgaccttgtgatccacccgcctcggcctcccaaagtgctgggattacaggcgtgagccaccacgcccggcctatccttttttttgtttttgagagggagtcgctctctggtcacccaggctggagtgcaatggtgctatcttggttcactgcaacctccgcctcccgggttcaagtgattctcctgcctcaacctcccaagtagctgagattacaggcacgtgccactatgccttgctaagttctgtatttttagtagagacaaggtttcaccgtattggccaggctggtctcgaactcctgatcttgtcatctgcctgccttggcctcccaaagtgctgggattataagtgtgagccactgtacctggcctgtagcatttatattctatttgcactttggtcacttaactatgtgaccaatttgtaactatttaacttatataagcaaccagcgtgtctcgaagaaaacaggaagaagtaaatttttccttcaaaattttgactttgctcctgatcatctgtgaaaggaactactcttagcttccaaaatcggaaaggtcgggagttaagatttaagagggaagattagcaaatttctggtactccctgaaagacacagttctcaaagtagtaatcatttctttgatggggatgagaagtgtttttctttctctcttctctttttttttcttttttcttttcgtttcttttctcttttcttttccttcttttctttctttcttctctttctttctctctctctctctctttctttttctttctttctttctctctttctctctttctttttttgagacacagtctcgctttgctgcccaggctggagtgcagtggcacaatctcggctcactgcaacctccatctcctgggtttaagcgattctcctgcctcagcctcccgagtagcttggattacaggcagctgccaccacgcccagctaatttttttgtacttttagtagagatggggtttcactatgtgggccaggctggtcttgaactcctgacctcaagtgatccccctgcctcagcctcccaaagtgctgggattacaggaatgagccactgcgcctggctgaaaggtgtatttcttcaacactaaattgcatttctgatctcagtttttaagagagacggatataaataagagaaagagaacacacattcaaggtgccaaacaattgatttgcacatatagtggcccttgaaccactcaggggttaggaatgcctacctaccctccagtcgaaaatttgtgtgtcacttttgactccccgagaattaactactaatagcctactgttgattgggagtcttaccaataacataaacagccaattaacacatattttgtgtgttatatgtatcatatactatattcttacaataaagtaagttagagaaaataaaatgtattaagaaaatcatgaggaagagaaaatatatttactattcattaagtggaagtggttcatcataaaggtcttcattcttggtgttttcatgttgaatagaccaaggaggaggggaagaaaggggagggtttggtcttgctgtctcaggggtggcagaagaggaagaaaagccctgtgtaagcgcatctgtgcagttccaacccgtgttgttcaagggtcaactggtatatgtttggaaatatagtttggaagctggggaaaggggtcagccttgctctgtaactaccacacttcctgtatgtgtctgcctttctcttttctactttttactttccactttttattttgaaaaatttcaaacccatagaaaagttaacagtacaatgcatactaatatgtccttcatcgggatttaccaattactaacattttgccatatctgctttgtctctttgtgtgtgtgttgaactgtttgaaagtaagtagcagacacttcaagcttaaatacttcaacatgcagctcctaataataaaattatcctacaaagccaaaataccattatctttttttttttttttttttaagacagagtctcattctgacatccaggctggagtgcagtggcaccatcttggctcactgcaacctctgccttctgagtttaagtaattcttctgcctcagtctcccaagcagctgggactacaggtgcacgctaccacaccgagctatttttaatagagatggggtttgccatgttggccaggctggtctcgaattcctggcctcaagtgatttgcctgcctcggcctcccaaagtgctgggattacaggagtgagccacctcgcccagcccaaaataccattgtcacatctatgaaaattaaccttaatccaataatatcatctaacaaacagtttacatttacatctctctatagctccccaatatttttttctcattttctcctcacctgtcatccagaatacaatgaagtttcatgcatggaatttggttattctatttctttagtctctttcaatcttaggagcatgctgtgtccaatacaggagccagtagccatgtgtggttatttacatttaaattatataaaatcagctgggcttggtggctcctgcctgcaatctcagctactcagggaggctgaggcaggaggatggcttgaggtcaggagttcgagaccagcctgggcaacatagcgagatcccatctctaaacaaattttttaaagtaattaattaaaataaataaatgtaaagaccagctcatctgttgcctagccacacttcaagtgcttagcagccatatttggctagcagttactatattgaacagcacagacataaactagtttcatcatcacagaaaggtctgttggacagtactgtctataacaatcccttgcccttttttttttgactttctttttagagtccatgccagttgtcttacaggaagtcgcatatcctggattgtctgtttattgcctcaagatttgatttaagaaacattttgggcaagagccccacacagaggatgtggtgtgcatcttagtatgttgctgatgtcaggtagctattagtgatgcctacactatgaattcaatgaacacttgttgaagaaatgatctggtgccaggcaatctcctaaggacttgggagcttgacttcaaataggagagagacagcttatataatctccagagcctccaacattgtcctaggagcagagtggaaaaatgctttgtaacatgaagggaagactgaagtgacatagcaaatggcccagcagcagcacagaggagagggacagacccagagaagggtgaggtcaagaggctacagctgttcctcagccccaacccccagactcacttcgatgatcataactttttggctgttgctttggggaggggcaggcagcttggtgaaatgcctgtgacccagctaagcattcagctggaagacttcgcagcaaggtgcccaaggaaaccctcaggacagagaggctggcaagttcaaagggcagcctgccagtcattcctctgctggcccgtgccaagggtctaggccagatttgggcctgggagtatctagggaaaacatcaaactatagttttcactgccttggttgtcacatttgcctccttctgtggctaccctccttccaccccaaataaaggccagggaaagaagacaggaaaaaagtgaaaactaaagagaaaattttgcttcaaagaactggttgtgtggttcccaactgtccatatggcacaggaaagtctcatctgtgaaacaaaataaagttcccttccaacacagacatgactgttctaatttcctatgttatttcaactctctaggaggtgagaaaagcagaaattattgcacccataggccatccttagttatccactgataacctgcccctccttgccaagaacttggaagtagcattgtcctcctacccctctcaaagataaactgtgaaatccacatgtaatgagaggtgcccaggcaggaggtgacattgacccaaggtataaacacacctaaagaaggaatgcactgatccaaagaaaggtctcagaggcaaagaaaggagactctgaaagaattctggcttcacttctttgggctctgtctggcagagggaccagagtcttacaagaatatctggccctctgtcaggtatccctattgtgcagactcatgcagccaaatataacaaggcctggcgcctgctggacttttgcgttttaaaactaacttctctattaggattcctgactttccaggtactttctgatcatctgccttcccttgtggcttgcttccaggagtgaatgtgctggtcaggctgacgtgtccgtccagtccactgaccagctggcatctggtcttatgcacaggcctctgggggtgtgtgggtctggcagcctccttgagtgggatgacatctgaatgggactaggtttctgagcctctgaggatgcagctggactcagggtcatagttggcttagcttagccatgtcatagccttcgcccagtggaagcctagctgtgaaacaggctggtcctcctcactgctcagcgttgtccagcttcagctgcacccatgtcacagatggataaaacccagcatcggctgggcttggtggctcacgcctgtaatcccaacactttgagaggccgaggcgggcggatcacctgaggtcgggagttcgagaccagcctgaccaacgtggagaaaccccgtctctactaaaaatacaaaaaaattagccaggtgtggtggcgaatgcctgtaatcccagctactcaggaggctgaggcaggagaatcgcttgaacttgggaggtggaggttgcagtaagtcgaaatcgcactattgcactccagcctgggcgacagagcaagactccatctcaaaaaaaaacaaaaaacaaaaaccaaaaacgaaacaaaaaaaacctcacaaaaaaacccagcatcgctccagggctatccacttcttcattccccagttccttcatattattaccaccactaattcaacccacattttatcatcatcatcataaaagcttctatttgtcgaatcttctgtgtgcctaacaaccccacagagagggcattattgttccattttggggaccaaaagaggctaattatggccacgagctgagagagctgggatccaaatctattactatgtctgtctacctctaattacaactatttttaaaaattaagctgggtgtggggatgagggaggtttcccagaagagtacagcatccttagcatgttttctgagtttcctcattccaaaggtggaaaacaggacccctacttactgaagtaaaaaaaaaaaaaaaaaaaagaatctgccctgattggcgaaggcagcctggcagttgtgtctggttggagaagcaggagaaattctaggtaagccctgggtcatctcagaggattctggcagccagctgtgaccctgatacagaaaaaagataacctagatgttaagctaagcgagagatatagaatgtagaagcatgagcagaagcatgagtgggcacatgatggactattctggctccacaggatgggagttatgagggcgagagatcagtggccttgttcttggcttggacgtgggtcccctaagagcacttccggccatggtgacatctttccccgctaccttcttgagcctgtgtcgaagggtggtttggtgtgtggcctgccaatcaggagactgtagttaatattccgtctttgacacctggggcaggtcttaaagttaacctcttaaagctttagtctccctttccatggacttcgaattcctaaaaaccacatactttatttctgagtaatttgtgaagtagttaacaatttaggtaatatgattgaaagttatgcgcatgacagcctgtggccgagtaaaagacagataaacatgtgggtgtcccaagaaggccgcaatttggggctcttctaatgcaatgttctctatacaattgttcaacatttttttcacttaacatttgaatataatacaaaatatttatgttcaaaacaaggactgtatatcacataaatatgactgaataggacataactttttttttttttttttgagatggagtctctctctgtcacccaggctggagtgcagtggcacgatctcggtttgctgcaagctctgcctcccgggttcacgccattctcctgcctcagcctcccgagtagctgggactacaggaacccaccaccacacccggctaatttttttattttttatttttagtggagacggggtttcagtgtgttaaccaggatggtcttgatctcctgacctcgtgatccgcccgcctcggcctcccaaagtgctgggaatacaggcgtgagccaccgcgcctggccaggacagaacatttaaacttatttggatgtgtttttcatttaacttaaaaaaatcaccaatgactagataatattagtcattcatacttaactaaacataaatatgactgtaaagtctttgaaattatttttaaacattcttttttggttggccaagctgtcttcacttttctgcaatttctttttctttcttgagttattaagatttttgtgtttttgaaaagagagtctcaccaaattgcccagactagacttgaactcctgagctcaactgatcctccggcctcagcctcctgggtagctgggactataagctcataccaccatgcctggctgtagagttttttttttgttttgtttctaatcattcaagccagacattttcatgggtgccatattaaaatatttcatatttagataatgtaataaaaatacagtacagtaaacagcattatactatgcattattcggtttctgaagtttagctaaaggagacaactaagttcaggagactgtcagctgactgacctctgaattggtagtgctgcctgtaattatgttataaaaataccatcagagataggctggcgccttggagccatgactttaaatgtccattggaagatactatttcagtaaacaattaacgttttgcagtcatgtatagtgtctcataagcaaaactgagataacaggcacccatttttctgatcgttttagcaatgttttatattccttataaaggggcaccatggccagccatttcatctggctccaggcatagaaggcacgcactgggctaagaaacctgggtgtgaatatatgacctggggcaagacatttaacttttctctgagcctcagtttttctcttgcaaaatggcaataatatctatctcatagcgttattagagaaaacattgatgttacaaatgagtctatcacttaaaagtatatgtatagtatactatatagtgaaacactatataaataataattaacaagcaattatcctctttccattaacctttactagccttataaacattgctttgaagagttagtactggagcacaggctgtgataaaaggcagatttttgagactggcaaatgttctgcacccagtatctgctcaatacttttgtgacatatcccatgggggcatgtcctgggtgggcagtggttcccgacacaggctttgtagtcagagatacctcagtggggctgtgctctgactctgcctttctgtatctgccatctcagaaaaactgctttgtcacaaatacgtgcgtctcataaggttgtgctatcaacgtctgcgctcccaactccagtcatacagagctatttgcagttcccaaaagcatcaggcttacttccttgctcagctcctggttccctctgcaggacggctctttctcctattttctgctaggctaactcctattcttctcagcttcctccaggatgtccctgactcccaagccttgatcaggtgcccttttcattggcccgctcccttatccaccctgaatttatcccatggccagcgtactgacatgacctagtcactggccttcgtccctcccacactgtagtattgattaggatttttgggtttagtatataccaggcacggagcttagtgctttgtttattatctcactgaggtctcataatgatcctatgaaataagtattagtactgatgaggaaactgaagctcagaaagggtgaatgatttgcccagggttatacaaatacaggcagaagagctgggatttgaaccaaggcccatctgactccaaaccctttgcagtcagtctattataagtttctaagggcttaaaggtgaacggtgaagacacacaggaaatactcaacaaataagagccgtcattattttgacccagattgtaagcctcggtagggagggaatcttaacccataaatgcttggacccatagcacaatcccccaacagaggctgagttaacacatggagaccagagtacaacctcctcgagagcaaggaccctgcatctagcttcttgagtgtgtccccgtgcaccagtttctcaataaatgcctgttgttttttcttttttttttttttttgaggcagagttttgctcttgtcacccagactggagtgcaatggcatgatgtcagctcactgcaacctccacctcctgggttcaagtgatcctcttgcctcagcctcccaagtagctgggattacaggcgcccgccaccacgcccagctaatttttgtagagacggggtttcaccatgttggccaagatggtctcgaactcctgacctcaggtgatccacccctctcagcctcccaaagtgctgggattacaggcatgagccgctgtgtctggcgatgctgtattttctatcacacaatctctgcattttagagatgtttcctttttttttttgagatggagtctcgttctgttgccaggctggagtgcagtggtgcaatcttggttcactgcaacctctgcctcctgggctcaagtggttctcctgcctcagcctcctgagtagctgggactacaggcacccgccaccacacctgactaatttttgtatttttagtagagacggggtttcatcatgttgaccaggattgtctccatctcttgagcttgtgatccgcccgcctcggcctcccaaagtgctgggattacaggcgtgagtcaccgcagccggccgagatgtttcatttcttgtcacactttggcccctttctactcctaattgaggagagggtaaggcctacagaggggcccaagacaacagttgaagctgctttttgatgagacatacaggaaacaccaaccatctaaataaacgtcctctttattttaccaaatataatttatcagttaagttgacatttgtcaattcagttatagtaactataaataattctcttaagacacagttctgtaactttttaaggatacgagagtaaaccaatattgctccttgcagccaggccaaaagtacatgcagttggtacaatcggggaaaagaaatgaaacttccatgaaagtcaccttcattttctttccctctcaccctacagtcctcctctgctcactcagggcctggggcatgcctatctgtctgctttttaggcaaaggaggtcactccagagtcttctgggactgcctggccaaattccagagatgaggaaggggcgagtgactggggtaggggtggctggagaccacagggacacagccttaggggcagaggagttggttttgatgcctgtacaagaagaatctgtgtgtaagtattttttgaggtggaggaaaagatgaaaaaagtccagagggaggaggaaaaacaagcccaggctggtgttaatgaattctgttggacacaactccaactagaaaacctctaaaattccttccaattctacggttctatgattccagaaggaggcctggaggtctgggtagaaatggagggagagaaaatatggtctctggaggtctagggcaggttcctgggataaggtgcagtgttggtagaaacaggatcattgcctaagccttcccttggaggtgggcccttgaggctacagatggaagggtttctgtagaagcttctgagagagaagttagaaaaagcctacatccaaatccccagatctgtacacgtgtgactgcggatggaggctccagttttctcccaattttgtgctaggcagagaaaagtagaaacaaccagatgatgtccaccctgctagttctaaatcctcttttgggtgcttggtaaggagaggtggagggaagggaatgtgaggaagggtcgtttagggaaataaatactggttgagcaatggggcggtggctctagctgtggtcagcactgcacagagtaggggtctggaaaggagaaagaggcagaagaatctggcttgaagtagatgcaaatacttacaacgaggaaactttctctgccagattcaaaggggcacatggcctttgtaacctggagaatgaggtgaggttagagctgtgtttcccttaccactggcttatcagtgcctggcacagtacctaacacatagtaggcactcaataaatattgctcaaagaatgtttcagaccatgcttgtctgcaggagagctcatcttgcggaggctgcatatttgctaaatgaacgaataaatgattggtgaatgtttgtgggtagaagccaagaaagaggaaaactgacctctatggcatgacagaacgagtaattttaggaagtgacagggtccaaggtgaccaagtgattatgtcctcaggagaaatggcagcaatgagacacctgtggttgtcctcaacctccaaaccattctccacatacccatgacctgaccctaatctcaaaacccaacctggcaagctctggggaaggtagtgcttagagacaatttgagatgaaggttgaagagagacaaagaatctgggcccagggagacaaagtcatttgggcccagggagaatgtggattttggggaaccaataggtggacatgggtcaacagggagaagagtgcactgttccattttttcctggatatgacaatcaactggaaatgatcagagggaggggttgttgatgttgaccaggccattgaacaagaggcatgtgcacaaattgaaaagtcagtccaccttactctttctgcgagtgggaacgcttaggtccagagggcaagagaacagaactgggatcacaggggcctggagcaggtgtctcctgtccagagctttgaagttggtccacttctacaaaagtatgtctgtgtttgggagtgttacttattcttctgtccctctgttcaaccaaaaccaaaaataaaacaaaacagataaaaagaaaacaaaaccaaaaatccagagcccacttacaaagggtttctcattagggccaagacaggttgctaaagccaaaccccatgtccccagattccagacaaaactcccctgctccagtccacatcacctggaggcacccaccatgaaactgcacttggtgattgtctcaaaaacctacttgtactgcttatctcaggccatctgtgtttcccaaattcttgctatacaaacttggctcaatgtataaaaattcccattgaaaataatgagaatttggtatcaaagtgaagtcctagaaagaggtgggagtgtggggtggaggagggacaggggaacaaaagaaaaatttcaaatagaaagtgcagagggatggggaaaatgttgagtgaccaagctagtccccgacatccgtgtctcggtcccctatgagccagagaacatggaagctgagtgctaggagcccagtgccaagcaggtcccccagagcagtcaagtatgggatggagaagttgtccgggtccaggccccggccccacatccagtgcaccatccagtctgcgatgtacaggagaatcagcacctggggagacaaaagggcccagcctatagccatcctctctctccagggggagccagaggccacatgatcagacccattcagtgcatcacagggcttggctggccataatccttactttttaatcttcctctttccaccccagcaacctctctgtgtttctccaccccacaattaccactttgagcagacaacaggcacaataagagctctttagaaaggaagatgctgctacgacccagggtcacccacatcagcattatattctgctcccaagtttaccaaacaaggagcttcctgacctaaatcctacttgttgcagaaactcagccctcttgcctctaactctgggtcacctcattctggggtcactccaattcctgccatgttggcctttccaggagcatggcagggggctggctgctggagtcagcttttcctaaagggatgtcttctctcggcagagtggtataaggatagtgtttgaagctgctgctggcggttgtcttaagtaacagatgatcatcccaagctggcttcctcctgacccttttcattctgttgttgtggcttttcattccattcttttccattgtttgggctcaaagaatgcaagtttattttaacattagtcctaataaagttgaattgtgaataagtcacctcaatattaatataaagcagacaatgcataccaattcaaaatacatttgacatgatctgtggctttgattttatctgtgttcttgcttaccttctattaatacagataattaagaatgactcagatcagaatctcgctagtgggcccaggaccagcagcatcaacaacagctgggtgcttgttagaaatgcaaaatctctggacctcttgagtcagagtccgcatttaacaagatttacatgcgcttttaagttggcgatgcccttgatctagaataccacggtggggcaggcctgaatctcctagaatctgcacagtgcctgacatttgggctccctaaatgactgcatctgcgtgagaatgaaacagattctgacggtcaagctctaatacagtcagtcatctgggaggttttacccttgactatactttgtaaatactgtggtatgaaaattctgccctaagggatccagatgcgggaaccacagcccttaagggatccagaagccagaactgatacctatttttaggcaatcttggttgctctcctgtcctctctctttttttttttttaaattttaggctctgcctgagagaatcctgccctctctccaaggaagccagagatgactcttcacattctcccttgctctgcacacagctgtcttgtgctaccacggccttggctcccctaccttccataacttcacaccctttccagcagctgcagaagggtcccaaataaagagcatggccaggaggcctttgggacatgccctaggaagggaatggtagcagctgtcctcacattccagcttcttgagcaggccccaggacacacagctgggaggaggtggcaaagggatcaataagagcctttacaggggatcaagtgtcacgctctggccctccacagatctagagaggacagcagaggcaagaatgtctccagggtattcatcatgggtgatggcactgaggctcatcctttccaattcaggccaagggatgagctgaaaacctccaccacagacccctggcatatccacccccatcttcccaccacgtgctgcactggaacccactagcaatggaatgtggcagcttggctaactgctgcagggcaacagcatatggctgattctcagccccgcccctgccaagatgtccgaacacaacctttctaaagctgggggtgagggggctggagggataggtgttaatcaatacaggactggcgaaataaaattatggtctgtgtatcacagaatatgatggagctgtaagaaaatcagggtgttgttctctttatgtattgatatggaatgatctcaaagataaacttaaatgaaaaatgcagggtgcagacagtgtgtacagtatactacatgtgtgtaaaaaagaggaaggaaataagaaaaatatatgtttacttttataaatatagaataggtttgaaggacacacaagaaagggataatactgatggtctgtgaaggagagaaacagatggctgtgaagaagaggacagaaaagaagacttttcactgaggtttctctatgaaccttaaaacatttttgaactatgtgactattcaaaaatcaaacctataaaaatttaaaatgtaataataagggtggatctagctgtaaagggatagcataagggagccttgtggtgatgaaacagttttctgtattttggttatagtggtggtcacacaaatctccacttgtgataaaaactgcatagaacgaacacacacgcacacacacacacgagtgcatgtaaaactggttcaatctgaataagcactgcagattgcatcaatgctaatttcctgattttgatactgtcctaaagttatgcaaaatgttattttcccatggagggaaattgggtaatggtatatgggatttctgaaccttttttttgagaacttcttacaaatctgtaatgatttcaaaataaaaagcttttacaatgtaataatacaagaagggagaaagtgtcatggtattatggaatggcaaggctacacaggatccgacagattatctagtgcagtggttttgacagtttttcaagctatgggatgctttatgcaaatgaatttcttgagaaagctcaacatgcaaaacagagccatgtggagctctgtggccagtggggttggcatgcaaaccccacaggctcagcatcctacaaccacctgcatgaaaactaccacccctggtccattcctctcaatttacaactgtatcgctgaggatcagggtagtaaaagaacagggtcaaagtcacacaccatgttggtgactctactggaactaccatctgttctcctgcacccttgtctggtgtttatcagctgccctgacacagagaaagaggaggttgagtgtctaagaggccaagtctggcctcctctcccatccctgcagggcatcctggctccttcccatgcccctgctcctgccactttgtacctggagcagtgcagctgtcatatagaagatgatgaagatgagtgtgagggtggtgtgcccgccctgcatacagctgatggtgtagaggaacaccaggtgtcctgggaccacgaggaggaagaggacccgggctgagcgagaattcacatctggaattggggaaaagagggtgtaaagaggaggggaggagaagacctggccccagaaggcctttcaaagtcaggagggacggcaccataccccagggcaacagacagatgaatgtctctacttctgcatcctgtggtctccaacccctagggtgctccaggaaaagacagccctcctgcctgggctctgcccttcagaacagctggcacagcccagcagagaaggagaacctgtggatctggggccccagctgtctcttaagtgaagctcactgacagtaggcccactccccccagggctgggaggctgggaatctgccgttaccagggctgaagaaggtggtacaaggactgggacagcggcgaggagcttgctcagagttctctccgggcattccattcatgtgcaggaaggtggagatgcggctggcctgcactgccaccagattgcccccaacacctgcagagacacatacgggcttagacacagacagaggtcagagggaggagtgggaacaaaatgatcttctcactctttgtcttctatctatagaggcactgtcctctgtcttaatttagggtctatgtgggcatcacccattcaccagtccccaaaagaagagtaaggcactaagaaggaagacaaagacccctgcttccagtgcatcttccagcctcccccatcctcccctctatggagatgcagcagttccatgttcccctggcaaagctgtgacagtgccggaaaggatacgtgcagatctgcagactcagagagcctgacttctccaccagtagagcatgggcacctgccttcctacacagctgaggggatgaagccctgccttgcctcaccgcctcacctcctctccaatgctctgagcagacccaggcatcctatggtcatatgctgattctggtaaccagtttcaaggatcaggtttgagctccaaactctggaatctggtatctccgccaggacctgtgctgatttctctgttgccctcacatcccaacctgctccctgctcttctcagccttgctctgagctctgggggactggtctccacagactgcattacccagtctcccttgctggctgcttccactgtttgttcagtgggaggcaacagcaggcaaccagagggcaggtggagagagagatcaggtatttctttcccaatccctccctgcttttcagcattggcttccccatgttgggggcaaagacagagctttcactggactcctataatgctattccctcgttactatggtttgaatatagtttgtccccaacaaaactcatgttgtggcttggtccccaaatgtggtggtgggaggtggtgcctttaagagtgaataggttattaagatggattaatgtctttcttgggaaaggtatagttcccatgagagtgggttgtcataaagcgaggtttgcctctcttgttttgcccattttgcacatgcccagttttccttctgtttctccatttggatgtttggatgcagcatgaggccctcactagaagcagctgctcaatcttgaacttcccagcttccagaactgtgagctaaataaacttcttttcgttataaattagccagtttcaagtattctgttctagcaacagataatggactatgatactccccttgaccctttaggagtagaggcttcccattgctgctaatctctcggtgcctcaacatcccttatctgtccttttactctgctcccacctctgtaagcagtcccttcattaaggtcttgaaccatctgagctagattctcgtctgctggaaccctgactgatacagaaaccaaccccttaagtcctcttctcctgtccctttccttcccccagccctgccctctgatagctgatgcccagacctcaccattaatcacaggcgtgaagacagccatcccagcaaagttggggtctgagacagtcttgtccaagatgaggcctcccacactatagagacataaagacaaaatgacgcaaagaccactgaagggttctgccttagtctctgggatgagaggtccaggcccacctatccttggagatgaagggaagcaccatggctctcaggagttcctcaccatccagtccttgcctcccttgacaggattaggtgctgctcataacattctgactgggcacagtgactccagaacaagctggtggtactgggtcaggcaaccacctcctgtacctgccctctaagttggccggaggagcagcctgcaggactatctgcctctgaggacctctgttgttctgcccactcagcatttacttccctttctggtgatagcactgggctcctccacagggaaccacctctctcaagctcagtgactgtggctcaggtgacaatgcctcaatgatagctaggctccaggtccatccaatcagaggattgcagccccaaggccacgctgactggtttggagataatcatgtcaccagatgagaagcagtggaactctattctgggactttgtggaactgttgggggaagaatctctcttcccactggaatttgtaggagtaagaaaagcataaacctgggctgtaggccatgacagagaagagcagagctaagagtcacagagtactggggccctgatcttaggtatgtcgctgaattcagctgtgcctttttggttctccaggccaatacattctgccttggaatgaaacccagttcagatggtttctgtcattttcaacagaaggacatgtgactgaaacactaatgaacacatttctagggtctgacccccaccccatctctccagggtttaaaaagaagtctgtggaagggttggagtggggtaggagtggatactcagggccccagcctacctgctgatggccatggcaatgataacaggctcccagcccgagtacaacacctcccttgtggctggacttcgtcgggccagcaccacccagacaggcagcagggccacaaagaaagcacacaccagtgggtagatgtatcgccagtgatctgagagggcagaggtcagaaggagataagcactgtgtttccctaccctaagtttctccctggctcagcctgaaaatgtcccaacagatcaatagcaagactacactaaatgccagtaaacacattatcccatttgatcttcactggcagctcaggaggtaggtgggacaagccttttccattttatggatgaggaaaccaagggagagagctagccaggcactgagccaattagggacagagaccagaggacagagactctaggtctcttgattggagcccagaaaacaccatctcccacccgcttcttcattttgcaagcagatctaagcctctggttcctttcctttaccctttccacctcatccctccaagagaagtaagaatctgcaggaccacacaggaatatacttctgatacttttcccctgcccctgatgcctgcttgaatttgagatcagtacttagcttcaaatctctaagatcaggaattattacaacctgtgttcaaaccaaatagtttaagaacacagaagaaactcttgcacatttgcaaactactaccatctctcccaaccccacccaggactccaagaagccacactcttggtggctcactcagttccaggtagagtccccagctgatgcctgagagcagcgccaaggtgatgaggtcgcccaggctggcagcaatgggtgtggccacgttgtctgggttgatcccaatcttgcgagagccaatgatgactccaatcatgatcatacctggtgagcaagtgggaggaggggcaggcagggtgagaagagataaaggagtctcaacaaacaaaaagagagagtggaagtgccaggtgcagtgttctctggggcggcactccttactcctctatgccctccctttcttacccagtaccagggaggcaatgaaggctgtggccacgctgctagcacagagcaggaaggcgtgcggaatactgaagtggccatcagggatccagccaaagacgacggctgcgatggacgccaggaagcccaccaccgtggcctgcacctggggacaggagtggtaactcagaaagccctgagagcagtgggcttcctaagctgaggtcataagcatctgggcagacctcttcctggctggcagtagccccaggaggcaggctggactgcatggtccagtcctcccaggctggaaggatgtctttatttatttaggttcacaccagccactagtactgggcagtgcactctgcaggagcccagaacatgttactggctgaatgagtgtgcctctggggatgggagtgaggttcaacagagccggagacttccacccagagtcaaggcctgggcctcaagggggaaggctcccagtctgaacctgtgtggtctcatggggagatgggacagcagtggcacaggacatctcagcactcctgagtctgctcatattgccaggatctgctgggactcaaaggcacgtgcaccaccaagaactgagaaccagaatgggtgatgctgggccctcctcatcttgggcgttttcctgggtaacctagttacctcctagagctactctgggggaagccagctcagtgggatactggagattcactcaggagcctgctggggctgacctaagcctttcagagattcctgactaaggggaagcttagcccaccctctctggtccctgccttcttacctggatgagggccatgttcccagtgatcatccgccagagctccttgggtgtgtccatgtgtccaatgttggcctgggaaagggagggcaaggggctggagcttcaggctggaaaaggcctgaagctccatccattaggctcctgcctagatcatgaggcagtacatgtggcctaagactctgagagcaggacctgacagtcccggaaaggtgaagcaggatcagggaaactgaggtgaaagggaaggagctaaagctgggctcctgcagctgggtggggggttggaagggggtcccctaggcagtcgcctctcttcctctcaggacaccagctgagcagaggcaaattctatcctttgccctgcttatctgggcagcccattcctgcatgggtcagaacaacccagtccctgactctgaagccagcctgcgatcccagggaaggaaaggtcagctgctggtgcaggactgaggctccaagagtatttgggaaggagtgggtggcatgggccagaagtcgggtatggcaagtcagggtgggttaacttggatgccacttctgtctgtcaccttctctagactcttgaccctgcagggagatccctggcctcctgagttttatcatctcccacctccagcccagggccctgtatctgttcaggcccggaatcgtcacggctcacaactgtgggaggtaggaatgacgagcagctcctctctgtctgtttccttaaagaagagcaagctgccatgggtaaagggaatgggatggccggggggctgggggtgctgggagggcctggctctgctcccgcccagctgcaaagcaggggctggagatcagaggaggcccccatctgtgcgggtggaggaaccagcatgatgcctgcctgtcaaagctgcacaaacagtcacgaggtggttgagaggtagggggtggggcaggagtccaggggtggctgggacatccagaaaccaagcctgggaaccactttgggcagggagcccctgcccaggagcaggacacccagcctgggatctccctacacctgcccagccaggccctcccttcccaccccagccccacactccaggcctgggcagtggagaagggctcgtagccctctcccagtctctggctctgtgctgcccagagtcctctctgtgccccactcctcccagccaggatactcactgcagtggaaagccttgatgccagggtcatttccaggttccctttgagccccagcagcgcaggcactaggatgaagacctctgtcaccttctggaagacttcccagtgctacgaggtgaaaacagaacccaggaatttcagtgccccaaagggcgggcattgaggttcaacaggtagtctgagatcaggggctcgaggaggaaatagaatcagcagggagtgagcacgccagccacctttcctccaagaaccttggaaccaaaccaagcccatgattcttcaaacaacacaaccccccttcctgccacccagaaccagggagatggagagggtttctgccggttgggagactctcagtctggccctaccttttctgttttcctggaggtgggtggggaagggtaatggggacccacacagctgagctgccctgggctgcctgacaccccagaaatcctttgcaatcccccctcaaattgcaatccctggcccctttgccttcagtccagtttctctgttgtctcagctgtgaagagttgggctccacagggctggggccgaggctggggagattagagagtttgtttggtttctatctccaagggctttgggcctcagccacagcaactctccttctgaacaggctctgaattaagactgtggcccctaaacctctgaatgctggcctgcaagaggctttttatttctctgtgcactgccttacccccacacaccttcctcaatctctcagctaggagaagcaagtgtactcctgtaggaagagccctggaccgggagtcaggagacctgagttctagtcccaagacaatcaatcctggctctcctaccaatgtctttggttaacatctattaaggactgattgtgtgctaggctaagtgctctccatgtattttctcttttaatcatcttaacaacccagtaaggtaggggctatttttattctcattttgtgaatgagtaaactggggttcagacagtattccactagttagtgctaagaggactgcaggaaccaggactggctatttgaaagctactttacttgcaattgaaactgaggacttgcaaaaaggtttaggattgtgtctccctccctggccctaacagggtaggtggtttcttttatttgttttaagaatggaaagcctccaggtttggagagggaggaggaggcaggaggccaggcggatatatatgggttggtctgcgtatcatggctgggaggccaagcactatgtttggcaagggcactggaccaagagccttgggtctcctacaggagacagcagggatggccccctgcttatctccccagtacacctcctcacgtagaccggctggacaccttagacaagttacaagggcctcaagctcttgaaaaatgttcaattcagggaccagatcagatggtctttcaaggcaattccaacacccacactctgtcgttaaagatgagcagtggccgagcgcagcggctcacacctataatcccagcactttgggaggccgaggcgggcagatcacctgaggccaggagtttgagaccagcctgaccaacatggagaaaccccgtctctactgaaaatacaaaaattagctggtcgtggtggcacatgcttgtaatcccaagctactcgggaggctgaggcaggagaatcgcttgaacccaagaggtggaggttgcagtgagccaagatcgcaccactgcactccagcctgggcaataagagtgaaactctgtctcaaaaataaaataaaataaaataaaataaaataaaataaaataaaataaaatagataaaataaagttgagcaatactgtagattagtaagagatcacctcacactcattaggatggttactatttaaaaacccagaaaataatcagtgttagcaaggatgtagagtttgggctgggcatagtggctcatgcctgtaatcccagcactttgggaggccaaggaaagtggatcacttgaggtcaggagttggagaccagcctggcaaacatagtgaaaccctgtttctactaaaaatacaaaaattagccgggaatggtggcgcacacctgtaatcccagctactggggaggctgaggcagaagaattgcttgaacttgggagttggaggttgcagtgagccgagacagtgccactgcactccagcctgggtgacagagcaagactccgtctcaagaaaagaaaaaagcatgtggagattggaacccttgtgcactcttggtgggactataaaatggtgcagctgctatgaaaaacagtacggtggttcctcaaaaaattaaaaataaaactaccacatgatccagcaatcccacttctggatatttatccaaaagaatagaaagcaaggtcttgaagatatattaatatgcccatgttcatagtagcactatatgtaataaccaagaggtggaagcaacccaaatgtccatcaaggaatgaatggataaacaaaatatgcaaagtgtggtacatatataccatggaatatttctcagccttaaaaaggaaggaaatcctgtcatatgccacaacatggatgaaccttgaggacattactctagtcataaaaaacactgtatgataaaacactcagataaaaaacacttatctgaggtatccaaagtagtcaaattcttttttttttttttttttttcttgagacacggtctcactctgtggcccaggctggagtgcagtggtgcaatcatggcttcgggctccagccatcctcccatctcagtctctcgggtagttgggactagaggcatgcaccaccacacctggctaatttttgtattttttgtagagacaggggtttcactatattgcccaggctggtctcgaactcctgggctcaaaggatcctctcgcctcgacctcccaaagtgtggggactacaggtatgaggcaccgagcccagcctaagtagtcaaattcatagaggcggaaagaagaatggtggaagcaaggcgctgggggagcagggaaaagagtgagtgtttaataggtacagagcttcagctggggaagatgaggagttctggagatctgttgtacaatgaggtgaatatacgtagtactattgaacagcacacttaaaaaagggttaagatggtaaattttatgttacacattttttaccacaataaccaaaaagataagcaaggctatcagagggggtggggctagggcttgagaccaggagaggctgggcgctgggtggccctataaggcaagaacctctcttttcctgtcggagctctccctgtgtgaatggggtgggaggcctcacaggatcctggggaaggactcatttcactggggctggagcatacgcttgcctgagcttctggtctggccaagacctgggactctccttagggaagccccaccgtagggactaacaatggggaagagactgccccccatctcaacaacagttactgggcttccaggcagccaaaggatgagccagccctctccaaacactgaagggaagtgaatcccttcccaccctaagaccccccagagagaaggcagccccagtgagccccatctgccctggagcaacttggggactgttactcttggacacggctggtacataccactgaggctccagctccctgcagtctggccttgctctgcttcgcctcctgcttcctcccaaaccagctccagagaggggaaaaatccccctcttctcccctcccttgcgggctttcaaagctcctctcagagcacagcctcagagctcatcttcaccccaaaacaccagctccaccctgcttccaagctgccagctccatgaaaatctgacttctacaggtaggtgtatgtaatgtacatgtactcatagaaagaaaaagcccacaagaagactccacatgtatgcaagcaatgttttctgagctgtttgtaatgaatattgcttgcttttattattatttaagaaaaatgtataaagctcagctaagttcctctggttgctaccataagcaccccaaatctctctacctcccagcacaatgcaccctctccttatagctacaggaggatctacaaagtacggagtgttaggagcagtgggataagagacagacaggcaaggagagggagcagtcacagtaacagcccctatgcaaaagtcttcccgactcttacagaatatagcctggaacctcaaacgacctgaccccaggccagcaaagccccgagttggcacttgggtcagagaagccaattcctacacacatactttcttcacccacaaaccctctcaaagctgcagctcaggcagaaagcctctgacacatgggcatgcataggactctggaaagagatgctggaggctggagatgtggagccagcccaggaatcaaggtggccttaaggttaggagtagacaggatgggcaggggcagacagtgagtagctcttcttcctcctttggccaaattcagccccatcctgttcatccaggctaggagtatctgcccctgaagtcacacccgtctgccaagcagccacccacgccttcctgctctgatggggatgaaaaagggcatgttccaggaagtgctgccctgcttggaggtgaggggagcatctagattttaactacttctcagaaatgcagctcctcatctctttccttctctaaccttggtgtgaggggctcatggatccctggtattctgcaggtgagggaatagactgcctcccccatagccaaaatgaatcctgaggcacagcaatcaccttaagtctcgatcctcagtggtcctgccagtacctcttccttgcccttccaatgcgcctcttccatccttcacctactccaatccaagctcatacactgaccctgacctgccttcaagggttctggcctgagccacctcaggagggtagcagcagggaagaaagtcagagccaggaatcaagacattaagaagacttaaattcccagatacaagctttaggctccaggctggggagaatctgggctcctgtgggagaagctgggctggagctgatcttttagggtaaggactgggtcagatgagattacagtaaccccaggcttcacctgtctgaggcttttccaaaaggcatcctctaggtgtccaggaaagggctttagggcaacacctggatatacggtgcaggacaaagcaggagcaaagcaaatgggtccctgacagcaggcaggggacagagatgggaaaagcagaaggggtggtcaagtgaagcagataagagtgtcccgcccagggatgctgcggccacaggagcaggccaggcacaggaggaatacttccttcccactctacttccccaaggccacgcttgccatgcactttcatcgttgtagacttctgtatacacagcaggatctactttgttcaagatccttagcaggtgagtagtgagttaaaataaggacctgtcttaacctagctgggaattaaagtgcagatgggcacactacttcctgtcaccccatccctcacaaaggctgacagataaagggagtgagacatccggagcagcctaggaccaaactgggcagatgggcacaaggctcctgcagtgaggaggctcccatatcccaacccccttcagaagccaacaccaggccccagcctgcttcccttccagatgctgcaggaactttcagccatggttgggaagttagagcagatggaggtccatttatccttttcctactttgggccagcaccagccccttatttcactgcagatgctgctgtgcacatttacgggagggcagataagaggaggcagaaatgacccttctaggaagagagtgggttttctttttcttttaaattaaaattaaaattcaactttttatttttattttttttgcatctcgttggtgaaaaagaaaccaagttttctacagcagcaaggaaagatgggggccctggaccaaggagacatctgaaccaggcccaatatggactcctgctcagttgctccaagatgctggggacactccatagccagcttctccagatggccccatggtcttggggcactttcagattctcttactgaagtccatcttagcttatgaaggggtaatataggtgtgaatccttagaaaccatcccgctcttcctgaatctgagattgtcagtcccccttttactcccatggatgtggaataacaatctccctgtggtcccatgtctcggtccctctgcactcaccccctcctgccatctcactgttgccatctgcagggcctgctccagcccagctgtagcaggaaggctgggggaggaggacatggacaaacctgtcattgtcatccacaccaagtggaccctagctctgaggtgagctgaggtgccacactgagagcagctccaaaggttccctacccaggcctctcaatgtctccagctcatgggcctggagtggggatggggcaacacatcagaaactttggaatctaagtgtgtgggatgggtaggggtgtggtgtgtatgcgggggtccctccctaccccatctaagaacttttattcttgctcacttcagaagataacgctaattaatccagattctaatccacccagttcttcaaggaaagacaaagaaaataggctcctcgtagagtctttttttttttttttttttttttgagacagcgtttggctctgttgctgaggctggagtgcagtggtacaatcatagctcattgcgacttcaaactcctgggctcaagtgatcactcctatctcagcctctcaaagtgctggaattatacgagaatgccaccatgcctgactattttttttttttttggtagagacaaggtctcactttgttgcccaggctggtcttgaactcctggcttcaagcgatcctcctgcctcagcctccaaaagtgctgggattacaggcataagccaccatgcccagccagagtttttttttttttgagttggagtctcgctctgtcacccaggctggagagcagtggcacgatcttggctcattgcagcctccacttctcgggctcaaatgattctcttgcctcagcttccaagtagctgggactacaggtgcctgccaccatgcccagctaattttttgtatttttagtagagacggggtttcactgtgttggccagactggtctcaaactcctgacctcaggtgatccgcccgtcttgacctcccaaagtgctaggattacaggcatgagccactgagctcggccccctctccgagtttttaaccaactggtgaaccatggccatggcgaaggccacaggggttagtggtgtgggctctagggtcagatgaccagggacaagttacctaatccctctaagctacaagttccctacctacaaaatggagatgattatggatcctacctcatgggcctaccgaagagccccccaaatgcttccccactaccattactattatccagaaaataagacaactctcttcagttcacctctggaccctggctctgcaaccctttgtaggtatcaaaccagaatgcaacaacttcaagaatgagaactgaggccacaggaaaggaatagaagaggtgaagaaaaatgttaccctagtctctttctcctcctcctactgtcccagtcccggccctagggggaggagcagcccctagcaggaggaacccaaagctccaggctggcttcccaacctccatgtaggaacaaccttcaagataacagttttggggaaaggggaggcagtgcaaggcactttggcatgacttaaacagcactctcatgagcaaccaaaggtgcagggttcccctgaagggctcaagtcaaagttctccatgtgcacacactatcaagaaccaacccccttcagtctcccaggaca